European Patent Application EP 4 321 166 A1, published February 14, 2024. Title: Composition for inhibiting Biofilm comprising Lactobacillus rhamnosus. Applicant: VIXXOL CORPORATION Chr.Hansen A/S. The sequence listing filed with the application follows.

SEQUENCE LISTING (2 sequences)

SEQ ID NO: 1 - DNA, 20 bp, Artificial Sequence
  Forward primer
cgcccttaacagcagtcttc

SEQ ID NO: 2 - DNA, 20 bp, Artificial Sequence
  Reverse primer
gccctccgtatgcttaaacc